European Patent Application EP 4 545 966 A1, published April 30, 2025. Title: REAGENT COMBINATION, KIT, DETECTION SYSTEM AND DETECTION METHOD FOR DETECTING SMALL MOLECULE. Applicant: NANJING POCLIGHT BIOTECHNOLOGY CO., LTD. Application EP. The sequence listing filed with the application follows.

SEQUENCE LISTING (3 sequences)

SEQ ID NO: 1 - DNA, 55 bp, synthetic construct
  source 1..55: mol_type = other DNA
acgctgagttatcaacgactttttttatcacatcaggctctagcgtatgctattg

SEQ ID NO: 2 - DNA, 53 bp, synthetic construct
  source 1..53: mol_type = other DNA
tacgtccagaactttaccaaaccacaccctttttttgtcgttggctgagattc

SEQ ID NO: 3 - DNA, 22 bp, synthetic construct
  source 1..22: mol_type = other DNA
cgatctcagcaactcagcagcg